European Patent Specification EP 3 526 244 B1, published September 6, 2023. Title: PEPTIDES DERIVES DU PROPEPTIDE NTSR3 ET LEUR UTILISATION DANS LE TRAITEMENT DE LA DEPRESSION. Applicant: CENTRE NATIONAL DE LA RECHERCHE SCIENTIFIQUE (CNRS) UNIVERSITE NICE SOPHIA ANTIPOLIS BORSOTTO, Marc MAZELLA, Jean HEURTEAUX, Catherine DJILLANI, Alaeddine MORENO, Sébastien PIETRI, Mariel. The sequence listing filed with the application follows.

SEQUENCE LISTING (7 sequences)

SEQ ID NO: 1 - protein, 44 aa, Artificial Sequence
  Propeptide PE
QDRLDAPPPPAAPLPRWSGPIGVSWGLRAAAAGGAFPRGGRWRR

SEQ ID NO: 2 - protein, 18 aa, Artificial Sequence
  Spadine
YAPLPRWSGPIGVSWGLR

SEQ ID NO: 3 - protein, 7 aa, Artificial Sequence
  Peptide PE(22-28)
GVSWGLR

SEQ ID NO: 4 - protein, 15 aa, Artificial Sequence
  Peptide PE(13-27)
PLPRWSGPIGVSWGL

SEQ ID NO: 5 - protein, 12 aa, Artificial Sequence
  Peptide PE(14-25)
LPRWSGPIGVSW

SEQ ID NO: 6 - protein, 9 aa, Artificial Sequence
  Peptide PI-PE(22-28)
PIGVSWGLR

SEQ ID NO: 7 - protein, 7 aa, Artificial Sequence
  Peptide G/A-PE(22-28)
AVSWGLR